European Patent Application EP 4 523 701 A2, published March 19, 2025. Title: Adenoviral vector vaccine against respiratory syncytial virus, and preparation method therefor and use thereof. Applicant: CANSINO BIOLOGICS INC. Application CN. The sequence listing filed with the application follows.

SEQUENCE LISTING (6 sequences)

SEQ ID NO: 1 - protein, 505 aa, synthetic construct
MELLILKANAITTILTAVTFCFASGQNITEEFYQSTCSAVSKGYLSALRTGWYTSVITIELSNIKENKCNGTDAKVKLIKQELDKYKNAVTELQLLMQSTPATGSGSAIASGVAVCKVLHLEGEVNKIKSALLSTNKAVVSLSNGVSVLTFKVLDLKNYIDKQLLPILNKQSCSISNIETVIEFQQKNNRLLEITREFSVNAGVTTPVSTYMLTNSELLSLINDMPITNDQKKLMSNNVQIVRQQSYSIMCIIKEEVLAYVVQLPLYGVIDTPCWKLHTSPLCTTNTKEGSNICLTRTDRGWYCDNAGSVSFFPQAETCKVQSNRVFCDTMNSLTLPSEINLCNVDIFNPKYDCKIMTSKTDVSSSVITSLGAIVSCYGKTKCTASNKNRGIIKTFSNGCDYVSNKGMDTVSVGNTLYYVNKQEGKSLYVKGEPIINFYDPLVFPSDEFDASISQVNEKINQSLAFIRKSDELLSAIGGYIPEAPRDGOAYVRKDGEWVLLSTFL

SEQ ID NO: 2 - protein, 535 aa, synthetic construct
MELLILKANAITTILTAVTFCFASGQNITEEFYQSTCSAVSKGYLSALRTGWYTSVITIELSNIKENKCNGTDAKVKLIKQELDKYKNAVTELQLLMQSTPATGSGSAIASGVAVCKVLHLEGEVNKIKSALLSTNKAVVSLSNGVSVLTFKVLDLKNYIDKQLLPILNKQSCSISNIETVIEFQQKNNRLLEITREFSVNAGVTTPVSTYMLTNSELLSLINDMPITNDQKKLMSNNVQIVRQQSYSIMCIIKEEVLAYVVQLPLYGVIDTPCWKLHTSPLCTTNTKEGSNICLTRTDRGWYCDNAGSVSFFPQAETCKVQSNRVFCDTMNSLTLPSEINLCNVDIFNPKYDCKIMTSKTDVSSSVITSLGAIVSCYGKTKCTASNKNRGIIKTFSNGCDYVSNKGMDTVSVGNTLYYVNKQEGKSLYVKGEPIINFYDPLVFPSDEFDASISQVNEKINQSLAFIRKSDELLHNVNAGKSTTNIMITTIIIVIIVILLSLIAVGLLLYCKARSTPVTLSKDQLSGINNIAFSN

SEQ ID NO: 3 - protein, 535 aa, synthetic construct
MELLILKANAITTILTAVTFCFASGQNITEEFYQSTCSAVSKGYLSALRTGWYTSVITIELSNIKENKCNGTDAKVKLIKQELDKYKNAVTELQLLMQSTPATGSGSAIASGVAVCKVLHLEGEVNKIKSALLSTNKAVVSLSNGVSVLTFKVLDLKNYIDKQLLPILNKQSCSISNIETVIEFQQKNNRLLEITREFSVNAGVTTPVSTYMLTNSELLSLINDMPITNDQKKLMSNNVQIVRQQSYSIMCIIKEEVLAYVVQLPLYGVIDTPCWKLHTSPLCTTNTKEGSNICLTRTDRGWYCDNAGSVSFFPQAETCKVQSNRVFCDTMNSLTLPSEINLCNVDIFNPKYDCKIMTSKTDVSSSVITSLGAIVSCYGKTKCTASNKNRGIIKTFSNGCDYVSNKGMDTVSVGNTLYYVNKQEGKSLYVKGEPIINFYDPLVFPSDEFDASISQVNEKINQSLAFIRKSDECCHNVNACCSTTNICCTTIIIVIIVILLSLIAVGLLLYCKARSTPVTLSKDQLSGINNIAFSN

SEQ ID NO: 4 - protein, 595 aa, synthetic construct
MELLILKANAITTILTAVTFCFASGQNITEEFYQSTCSAVSKGYLSALRTGWYTSVITIELSNIKENKCNGTDAKVKLIKQELDKYKNAVTELQLLMQSTPATGSGSAIASGVAVCKVLHLEGEVNKIKSALLSTNKAVVSLSNGVSVLTFKVLDLKNYIDKQLLPILNKQSCSISNIETVIEFQQKNNRLLEITREFSVNAGVTTPVSTYMLTNSELLSLINDMPITNDQKKLMSNNVQIVRQQSYSIMCIIKEEVLAYVVQLPLYGVIDTPCWKLHTSPLCTTNTKEGSNICLTRTDRGWYCDNAGSVSFFPQAETCKVQSNRVFCDTMNSLTLPSEINLCNVDIFNPKYDCKIMTSKTDVSSSVITSLGAIVSCYGKTKCTASNKNRGIIKTFSNGCDYVSNKGMDTVSVGNTLYYVNKQEGKSLYVKGEPIINFYDPLVFPSDEFDASISQVNEKINQSLAFIRKSDELLSAIGGYIPEAPRDGOAYVRKDGEWVLLSTFLGGSGGSGGSKQRQNKPPNKPNNDFHFDVFNFVPCSICSNNPTCWAICKRIPNKKPGKKTTTKPTKKPTFKTTKKDHKPQTTKPKEVPTTK

SEQ ID NO: 5 - protein, 544 aa, synthetic construct
MELLILKANAITTILTAVTFCFASGQNITEEFYQSTCSAVSKGYLSALRTGWYTCVITIELSNIKENKCNGTDAKVKLIKQELDKYKNAVTELQLLMQSTPPTNNRARRELPRFMNYTLNNAKKTNVTLSKKRKRRFLGFLLGVGSAIASGVAVSKVLHLEGEVNKIKSALLSTNKAVVSLSNGVSVCTIKVLDLKNYIDKQLLPIVNKQSCSISNIETVIEFQQKNNRLLEITREFSVNAGVTTPVSTYMLTNSELLSLINDMPITNDQKKLMSNNVQIVRQQSYSIMSIIKEEVLAYVVQLPLYGVIDTPCWKLHTSPLCTTNTKEGSNICLTRTDRGWYCDNAGSVSFFPQAETCKVQSNRVFCDTMNSLTLPSEINLCNVDIFNPKYDCKIMTSKTDVSSSVITSLGAIVSCYGKTKCTASNKNRGIIKTFSNGCDYVSNKGMDTVSVGNTLYYVNKQEGKSLYVKGEPIINFYDPLVFPSSEFDASISQVNEKINQSLAFIRKSDELLSAIGGYIPEAPRDGQAYVRKDGEWVLLSTFL

SEQ ID NO: 6 - protein, 574 aa, synthetic construct
MELLILKANAITTILTAVTFCFASGQNITEEFYQSTCSAVSKGYLSALRTGWYTCVITIELSNIKENKCNGTDAKVKLIKQELDKYKNAVTELQLLMQSTPPTNNRARRELPRFMNYTLNNAKKTNVTLSKKRKRRFLGFLLGVGSAIASGVAVSKVLHLEGEVNKIKSALLSTNKAVVSLSNGVSVCTIKVLDLKNYIDKQLLPIVNKQSCSISNIETVIEFQQKNNRLLEITREFSVNAGVTTPVSTYMLTNSELLSLINDMPITNDQKKLMSNNVQIVRQQSYSIMSIIKEEVLAYVVQLPLYGVIDTPCWKLHTSPLCTTNTKEGSNICLTRTDRGWYCDNAGSVSFFPQAETCKVQSNRVFCDTMNSLTLPSEINLCNVDIFNPKYDCKIMTSKTDVSSSVITSLGAIVSCYGKTKCTASNKNRGIIKTFSNGCDYVSNKGMDTVSVGNTLYYVNKQEGKSLYVKGEPIINFYDPLVFPSSEFDASISQVNEKINQSLAFIRKSDELLHNVNAGKSTTNIMITTIIIVIIVILLSLIAVGLLLYCKARSTPVTLSKDQLSGINNIAFSN